European Patent Application EP 4 335 865 A1, published March 13, 2024. Title: Interaction between a glycolipid and major capsid protein (VP1) of sheep polyomavirus and, methods, kits and uses thereof. Applicant: Eberhard Karls Universität Tübingen. Application EP, filed September 7, 2022. The sequence listing filed with the application follows.

SEQUENCE LISTING (9 sequences)

SEQ ID NO: 1 - protein, 357 aa, Sheep polyomavirus 1
  source 1..357: note = YP_009134726.1 VP1
MAPKKRSLGQPAPVPKLIVKGGIEVLAVRTGPDSITEIEAYLNPRMGQPQNEDFYGFSDNVTVSDDFGSDAPPWKQFPCYSTARISLPMLNQDMTCDTILMWEAISCRTEVMGVNMLTNVHSAQKRVYENDREGTGIGVEGMGYHMFAIGGEPLELQFMVFNHRATYPAEATVIKNPGASSQVFDPNLKGTLTADGVFPVEAWGPDPFKNENTRYFGQYTGGTQTPPVLTFTNTQTTILLDENGVGPLCKGDGLFLSCADIVGFFTQHNKKMSFRGLPRYFRVTLRKRVVKNPYPVSHLLNTLFSNMQPTVRGQPMQGEDAQVEEVRVYQGVEGLPGDPDMVRFRDQFGQTNTVVGN

SEQ ID NO: 2 - protein, 293 aa, synthetic construct
  source 1..293: note = Recombinant ShPyV VP1 construct
MGSSHHHHHHSSGLVPRGSHMGGIEVLAVRTGPDSITEIEAYLNPRMGQPQNEDFYGFSDNVTVSDDFGSDAPPWKQFPCYSTARISLPMLNQDMTSDTILMWEAISCRTEVMGVNMLTNVHSAQKRVYENDREGTGIGVEGMGYHMFAIGGEPLELQFMVFNHRATYPAEATVIKNPGASSQVFDPNLKGTLTADGVFPVEAWGPDPFKNENTRYFGQYTGGTQTPPVLTFTNTQTTILLDENGVGPLCKGDGLFLSCADIVGFFTQHNKKMSFRGLPRYFRVTLRKRVVKN

SEQ ID NO: 3 - protein, 270 aa, synthetic construct
  source 1..270: note = core sequence of ShPyV VP1 construct
IEVLAVRTGPDSITEIEAYLNPRMGQPQNEDFYGFSDNVTVSDDFGSDAPPWKQFPCYSTARISLPMLNQDMTSDTILMWEAISCRTEVMGVNMLTNVHSAQKRVYENDREGTGIGVEGMGYHMFAIGGEPLELQFMVFNHRATYPAEATVIKNPGASSQVFDPNLKGTLTADGVFPVEAWGPDPFKNENTRYFGQYTGGTQTPPVLTFTNTQTTILLDENGVGPLCKGDGLFLSCADIVGFFTQHNKKMSFRGLPRYFRVTLRKRVVKN

SEQ ID NO: 4 - DNA, 44 bp, synthetic construct
  source 1..44: mol_type = other DNA; note = S95C_fwd
gctgaaccaagacatgacctgcgataccatcctgatgtgggagg

SEQ ID NO: 5 - DNA, 44 bp, synthetic construct
  source 1..44: mol_type = other DNA; note = S95C_rev
cctcccacatcaggatggtatcgcaggtcatgtcttggttcagc

SEQ ID NO: 6 - DNA, 30 bp, synthetic construct
  source 1..30: mol_type = other DNA; note = T61I_fwd
gcgataacgtgattgttagcgacgatttcg

SEQ ID NO: 7 - DNA, 30 bp, synthetic construct
  source 1..30: mol_type = other DNA; note = T61I_rev
cgaaatcgtcgctaacaatcacgttatcgc

SEQ ID NO: 8 - DNA, 34 bp, synthetic construct
  source 1..34: mol_type = other DNA; note = Q266F_fwd
gggtttctttacctttcacaacaagaaaatgagc

SEQ ID NO: 9 - DNA, 34 bp, synthetic construct
  source 1..34: mol_type = other DNA; note = Q266F_rev
gctcattttcttgttgtgaaaggtaaagaaaccc